European Patent Application EP 4 183 416 A1, published May 24, 2023. Title: Agent for treatment or prevention of muscle disease. Applicant: Mitsubishi Tanabe Pharma Corporation. The sequence listing filed with the application follows.

SEQUENCE LISTING (4 sequences)

SEQ ID NO: 1 - DNA, 446 bp, Mus musculus
  CDS (231)..(368)
agtgagcttttcgtccatggagagcagatggtgtttttgaaaggaagggcggccattcccaggactttggacttggctccgttgcacccctgaacagaaccaacgttgctaggagaacacctgtgccccagcactttggtccagcaagggcaggagaggagagctggaaactggtagagctgtgctacctgctacctcctgaggctctcagggagcaggagaatctgaacatgagtggcaagagctgggtactgatctctactacttcgccccagagcctggaagatgagattctgggacggcttctgaaaattctcttcgttttgttcgttgacttaatgtccattatgtatgtcgtcataacgtcctagcaacctgactttctttactccgtgtgtaagtttcaaaccaaatgcgagcaaataaagatctacattttaatctga

SEQ ID NO: 2 - protein, 46 aa, Mus musculus
MSGKSWVLISTTSPQSLEDEILGRLLKILFVLFVDLMSIMYVVITS

SEQ ID NO: 3 - DNA, 857 bp, Homo sapiens
  CDS (349)..(486)
agaccagtgagcctcctgatccaccaagaccatatggtgtttttcataaaagagagagatcattcccttgactttggacttcgcttattgaacccctggacaacggaatctccctctgtcgcccaggctggagtgcagtggcaccatctcggcttaccgcaacctccgcctcctgggttcaaacaatactcctaccttggcctcctgagtagctgggattacaggaatcaaggttgctaagagaccacctgtgctgaatacactttgttctggcaagagcagaaaactgagaagccgtgttacctaccactacctgggattaattcagggagcgggataattctggatatgactggtaaaaactggatattaatttctactactactcccaaaagtctagaagatgaaattgtgggaagacttctaaaaattttgtttgttatctttgttgacttaatttctattatatatgttgtgataacttcttagaaagctgacttcctttccatgtacatttcaaactgaattacagtgaataaaaatttgtattttaacttgttgagtgactcacattttatgacattgccaatttattctagaagccaacaggacactgcaatacaaacaacattgtgtattgtttagttctttatggtttatgaaacattcacatatactgaagtgaatttttttccccaaaaacatctatcctactgagtcatgaaacttctagatttttagccaggtgtggtggctcacacctgtaatcccagcactttgagaggcccaggtaggcggatcccttgagtgcaggagttcgatacgggcctgagcaacctgaagaaatcccatctcta

SEQ ID NO: 4 - protein, 46 aa, Homo sapiens
MTGKNWILISTTTPKSLEDEIVGRLLKILFVIFVDLISIIYVVITS